European Patent Specification EP 3 626 829 B1, published November 22, 2023. Title: Judgment marker and judgment method of Parkinson's disease. Applicant: KABUSHIKI KAISHA YAKULT HONSHA National University Corporation Nagoya University. The sequence listing filed with the application follows.

SEQUENCE LISTING (38 sequences)

SEQ ID NO: 1 - DNA, 20 bp, Artificial Sequence
  Designed primer based on Clostridium coccoides group
aaatgacggtacctgactaa

SEQ ID NO: 2 - DNA, 22 bp, Artificial Sequence
  Designed primer based on Clostridium coccoides group
ctttgagtttcattcttgcgaa

SEQ ID NO: 3 - DNA, 16 bp, Artificial Sequence
  Designed primer based on Clostridium leptum subgroup
gcacaagcagtggagt

SEQ ID NO: 4 - DNA, 18 bp, Artificial Sequence
  Designed primer based on Clostridium leptum subgroup
cttcctccgttttgtcaa

SEQ ID NO: 5 - DNA, 21 bp, Artificial Sequence
  Designed primer based on Bacteroides fragilis group
ayagcctttcgaaagraagat

SEQ ID NO: 6 - DNA, 21 bp, Artificial Sequence
  Designed primer based on Bacteroides fragilis group
ccagtatcaactgcaatttta

SEQ ID NO: 7 - DNA, 17 bp, Artificial Sequence
  Designed primer based on Genus Bifidobacterium
ctcctggaaacgggtgg

SEQ ID NO: 8 - DNA, 22 bp, Artificial Sequence
  Designed primer based on Genus Bifidobacterium
ggtgttcttcccgatatctaca

SEQ ID NO: 9 - DNA, 17 bp, Artificial Sequence
  Designed primer based on Atopobium cluster
gggttgagagaccgacc

SEQ ID NO: 10 - DNA, 18 bp, Artificial Sequence
  Designed primer based on Atopobium cluster
cggrgcttcttctgcagg

SEQ ID NO: 11 - DNA, 20 bp, Artificial Sequence
  Designed primer based on Genus Prevotella
cacrgtaaacgatggatgcc

SEQ ID NO: 12 - DNA, 16 bp, Artificial Sequence
  Designed primer based on Genus Prevotella
ggtcgggttgcagacc

SEQ ID NO: 13 - DNA, 18 bp, Artificial Sequence
  Designed primer based on Clostridium perfringens
gggggtttcaacacctcc

SEQ ID NO: 14 - DNA, 18 bp, Artificial Sequence
  Designed primer based on Clostridium perfringens
gcaagggatgtcaagtgt

SEQ ID NO: 15 - DNA, 23 bp, Artificial Sequence
  Designed primer based on Family Enterobacteriaceae
tgccgtaacttcgggagaaggca

SEQ ID NO: 16 - DNA, 22 bp, Artificial Sequence
  Designed primer based on Family Enterobacteriaceae
tcaaggaccagtgttcagtgtc

SEQ ID NO: 17 - DNA, 17 bp, Artificial Sequence
  Designed primer based on Lactobacillus casei subgroup
accgcatggttcttggc

SEQ ID NO: 18 - DNA, 20 bp, Artificial Sequence
  Designed primer based on Lactobacillus casei subgroup
ccgacaacagttactctgcc

SEQ ID NO: 19 - DNA, 27 bp, Artificial Sequence
  Designed primer based on Lactobacillus gasseri subgroup
gatgcatagccgagttgagagactgat

SEQ ID NO: 20 - DNA, 25 bp, Artificial Sequence
  Designed primer based on Lactobacillus gasseri subgroup
taaaggccagttactacctctatcc

SEQ ID NO: 21 - DNA, 25 bp, Artificial Sequence
  Designed primer based on Lactobacillus plantarum subgroup
ctctggtattgattggtgcttgcat

SEQ ID NO: 22 - DNA, 24 bp, Artificial Sequence
  Designed primer based on Lactobacillus plantarum subgroup
gttcgccactcactcaaatgtaaa

SEQ ID NO: 23 - DNA, 16 bp, Artificial Sequence
  Designed primer based on Lactobacillus reuteri subgroup
gaacgcaytggcccaa

SEQ ID NO: 24 - DNA, 19 bp, Artificial Sequence
  Designed primer based on Lactobacillus reuteri subgroup
tccattgtggccgatcagt

SEQ ID NO: 25 - DNA, 21 bp, Artificial Sequence
  Designed primer based on Lactobacillus ruminis subgroup
caccgaatgcttgcaytcacc

SEQ ID NO: 26 - DNA, 19 bp, Artificial Sequence
  Designed primer based on Lactobacillus ruminis subgroup
gccgcgggtccatccaaaa

SEQ ID NO: 27 - DNA, 22 bp, Artificial Sequence
  Designed primer based on Lactobacillus sakei subgroup
cataaaacctamcaccgcatgg

SEQ ID NO: 28 - DNA, 27 bp, Artificial Sequence
  Designed primer based on Lactobacillus sakei subgroup
tcagttactatcagatacrttcttctc

SEQ ID NO: 29 - DNA, 24 bp, Artificial Sequence
  Designed primer based on Lactobacillus brevis
attttgtttgaaaggtggcttcgg

SEQ ID NO: 30 - DNA, 25 bp, Artificial Sequence
  Designed primer based on Lactobacillus brevis
acccttgaacagttactctcaaagg

SEQ ID NO: 31 - DNA, 23 bp, Artificial Sequence
  Designed primer based on Lactobacillus fermentum
cctgattgattttggtcgccaac

SEQ ID NO: 32 - DNA, 26 bp, Artificial Sequence
  Designed primer based on Lactobacillus fermentum
acgtatgaacagttactctcatacgt

SEQ ID NO: 33 - DNA, 20 bp, Artificial Sequence
  Designed primer based on Genus Enterococcus
atcagagggggataacactt

SEQ ID NO: 34 - DNA, 21 bp, Artificial Sequence
  Designed primer based on Genus Enterococcus
actctcatccttgttcttctc

SEQ ID NO: 35 - DNA, 30 bp, Artificial Sequence
  Designed primer based on Genus Staphylococcus
tttgggctacacacgtgctacaatggacaa

SEQ ID NO: 36 - DNA, 24 bp, Artificial Sequence
  Designed primer based on Genus Staphylococcus
aacaactttatgggatttgcwtga

SEQ ID NO: 37 - DNA, 23 bp, Artificial Sequence
  Designed primer based on Genus Pseudomonas
caaaactactgagctagagtacg

SEQ ID NO: 38 - DNA, 25 bp, Artificial Sequence
  Designed primer based on Genus Pseudomonas
taagatctcaaggatcccaacggct